European Patent Specification EP 3 504 234 B1, published July 22, 2026. Title: HETERODIMERIC IMMUNOGLOBULIN CONSTRUCTS AND PREPARATION METHODS THEREOF. Applicant: Beijing Hanmi Pharm. Co., Ltd. Liu , Jiawang Song, Nanmeng Yang , Dongge Yang , Yaping Kim, Maeng Sup. The sequence listing filed with the application follows.

SEQUENCE LISTING (80 sequences)

SEQ ID NO: 1 - DNA, 22 bp, Artificial
  Synthetic
tggggcccagccggccagatct

SEQ ID NO: 2 - DNA, 27 bp, Artificial
  Synthetic
ataagaatgcggccgcgtcgacctgca

SEQ ID NO: 3 - DNA, 41 bp, Artificial
  Synthetic
atcgagtcaatattagggttagtaaaagggtcctaaggaac

SEQ ID NO: 4 - DNA, 44 bp, Artificial
  Synthetic
cagtcgataatattaagaattaattctcatgtttgacagcttat

SEQ ID NO: 5 - DNA, 37 bp, Artificial
  Synthetic
tagcctccccctagggtgggcgaagaactccagcatg

SEQ ID NO: 6 - DNA, 49 bp, Artificial
  Synthetic
tttggaggcctaggcttttgcaaagatcgatcaagagacaggatgagga

SEQ ID NO: 7 - DNA, 2773 bp, Artificial
  Synthetic
tgctggggcccagccggccatgagcgacagcgaggtgaaccaggaggccaaacccgaggtgaagcccgaggtgaaacccgagacccacatcaacctgaaggtgagcgacggcagcagcgagatcttcttcaagatcaagaagaccacccccctgaggaggctgatggaggccttcgccaagaggcagggcaaggagatggacagcctgaggttcctgtacgacggcatccgtattcaagccgaccagacccctgaggacctggacatggaggacaacgacatcatcgaggcccacagggagcagatcggcggcgaacccaagtccagcgataagacccacacatgccctccctgtcctgctcccgaactgctgggaggaccctccgtcttcctgttcccccccaagcccaaagacacactgatgatcagcaggacccctgaagtgacctgcgtggtcgtggacgtgagccacgaggaccccgaggtcaagtttaactggtacgtggacggcgtggaggtccacaacgccaagaccaagcccagggaggagcagtacaacagcacctacagggtcgtgtccgtgctgaccgtgctccaccaagattggctcaacggcaaggagtataagtgcaaagtcagcaacaaggccctccccgcccccatcgagaaaaccatcagcaaggccaagggccaaccgcgggaacctcaagtgtataccctccctcccagccgggatgagctgaccaagaaccaagtctccctcacctgcctggtcaagggattctacccttccgacattgccgtcgaatgggagagcaatggccagcccgagaacaactacaagacaaccccccccgtcctggatagcgacggatccttcttcctgtactccaagctcaccgtcgacaagagccggtggcaacagggcaacgtgttctcctgtagcgtgatgcacgaagccctccacaaccactatacccagaagagcctgagcctcagccccggcaaatgatgaagatctctagagctcgctgatcagcctcgactgtgccttctagttgccagccatctgttgtttgcccctcccccgtgccttccttgaccctggaaggtgccactcccactgtcctttcctaataaaatgaggaaattgcatcgcattgtctgagtaggtgtcattctattctggggggtggggtggggcaggacagcaagggggaggattgggaagacaatagcaggcatgctggggatgcggtgggctctatggcttctgaggcggaaagaaccagctggggctctagggggtatccccacgcgccctgtagcggcgcagcgcgcgttgacattgattattgactagttattaatagtaatcaattacggggtcattagttcatagcccatatatggagttccgcgttacataacttacggtaaatggcccgcctggctgaccgcccaacgacccccgcccattgacgtcaataatgacgtatgttcccatagtaacgccaatagggactttccattgacgtcaatgggtggactatttacggtaaactgcccacttggcagtacatcaagtgtatcatatgccaagtacgccccctattgacgtcaatgacggtaaatggcccgcctggcattatgcccagtacatgaccttatgggactttcctacttggcagtacatctacgtattagtcatcgctattaccatggtgatgcggttttggcagtacatcaatgggcgtggatagcggtttgactcacggggatttccaagtctccaccccattgacgtcaatgggagtttgttttggcaccaaaatcaacgggactttccaaaatgtcgtaacaactccgccccattgacgcaaatgggcggtaggcgtgtacggtgggaggtctatataagcagagctctctggctaactagagaacccactgcttactggcttatcgaaatgccaccatggagacagacacactcctgctatgggtactgctgctctgggttccaggttccactggtgactatccatatgatgttccagattatgctgagcccaagtccagcgacaagacccacacatgccccccttgtcctgcccctgaactgctcggaggccctagcgtgttcctcttccctcccaaacccaaggacaccctcatgatctccaggacccctgaggtgacctgcgtcgtggtggacgtcagccacgaggaccccgaggtgaagttcaactggtacgtggacggcgtcgaggtccacaacgccaagacaaagcccagggaggaacagtacaacagcacctacagggtggtcagcgtgctgaccgtgctgcaccaggattggctcaacggcaaggagtacaagtgcaaagtctccaacaaggccctgcccgcccccatcgagaagaccatctccaaggctaagggacagcccagggagccccaagtgtacaccctccctcccagccgggatgagctgaccaagaaccaagtctccctcacctgcctggtcaagggattctacccttccgacattgccgtcgaatgggagagcaatggccagcccgagaacaactacaagacaaccccccccgtcctggatagcgacggatccttcttcctgtactccaagctcaccgtcgacaagagcagatggcagcagggcaacgtgttcagctgtagcgtgatgcacgaggccctgcacaaccactacacccagaagagcctgtccctcagccccggcaagctgcagaat

SEQ ID NO: 8 - DNA, 69 bp, Artificial
  Synthetic
  misc_feature (41)..(42): n can be a, c, g or t
tcccagccgggatgagctgaccaagaaccaagtctccctcnnstgcctggtcaagggattctacccttc

SEQ ID NO: 9 - DNA, 66 bp, Artificial
  Synthetic
  misc_feature (44)..(45): n can be a, c, g or t
gtccacggtgagcttggagtacaggaagaaggatccgtcgctsnncaggacggggggggttgtctt

SEQ ID NO: 10 - DNA, 27 bp, Artificial
  Synthetic
tactccaagctcaccgtggacaagagc

SEQ ID NO: 11 - DNA, 52 bp, Artificial
  Synthetic
cgatccaatcgatggaagatcttcatcatttgccggggctgaggctcaggct

SEQ ID NO: 12 - DNA, 70 bp, Artificial
  Synthetic
caagggccagccgcgggaacctcaagtgtataccctccctcccagccgggatgagctgaccaagaaccaa

SEQ ID NO: 13 - DNA, 52 bp, Artificial; identical to SEQ ID NO: 11
  Synthetic

SEQ ID NO: 14 - DNA, 54 bp, Artificial
  Synthetic
  misc_feature (31)..(32): n can be a, c, g or t
ggccagcccagggaacctcaagtgtacaccnnscctcccagccgggatgagctg

SEQ ID NO: 15 - DNA, 63 bp, Artificial
  Synthetic
  misc_feature (35)..(36): n can be a, c, g or t
  misc_feature (41)..(42): n can be a, c, g or t
gccctgttgccaccggctcttgtcgacggtgagsnnggasnncaggaagaaggatccgtcgct

SEQ ID NO: 16 - protein, 232 aa, Artificial
  Fc1 sequence
EPKSCDKTHTCPPCPAPELLGGPSVFLFPPKPKDTLMISRTPEVTCVVVDVSHEDPEVKFNWYVDGVEVHNAKTKPREEQYNSTYRVVSVLTVLHQDWLNGKEYKCKVSNKALPAPIEKTISKAKGQPREPQVYTLPPSRDELTKNQVSLLCLVKGFYPSDIAVEWESNGQPENNYKTTPPVLCSDGSFFLYSKLTVDKSRWQQGNVFSCSVMHEALHNHYTQKSLSLSPGK

SEQ ID NO: 17 - protein, 232 aa, Artificial
  Fc2 sequence
EPKSCDKTHTCPPCPAPELLGGPSVFLFPPKPKDTLMISRTPEVTCVVVDVSHEDPEVKFNWYVDGVEVHNAKTKPREEQYNSTYRVVSVLTVLHQDWLNGKEYKCKVSNKALPAPIEKTISKAKGQPREPQVYTGPPSRDELTKNQVSLTCLVKGFYPSDIAVEWESNGQPENNYKTTPPVLDSDGSFFLLSCLTVDKSRWQQGNVFSCSVMHEALHNHYTQKSLSLSPGK

SEQ ID NO: 18 - protein, 232 aa, Artificial; identical to SEQ ID NO: 16
  Fc1 sequence

SEQ ID NO: 19 - protein, 232 aa, Artificial
  Fc2 sequence
EPKSCDKTHTCPPCPAPELLGGPSVFLFPPKPKDTLMISRTPEVTCVVVDVSHEDPEVKFNWYVDGVEVHNAKTKPREEQYNSTYRVVSVLTVLHQDWLNGKEYKCKVSNKALPAPIEKTISKAKGQPREPQVYTYPPSRDELTKNQVSLTCLVKGFYPSDIAVEWESNGQPENNYKTTPPVLDSDGSFFLASPLTVDKSRWQQGNVFSCSVMHEALHNHYTQKSLSLSPGK

SEQ ID NO: 20 - protein, 232 aa, Artificial
  Fc1 sequence
EPKSCDKTHTCPPCPAPELLGGPSVFLFPPKPKDTLMISRTPEVTCVVVDVSHEDPEVKFNWYVDGVEVHNAKTKPREEQYNSTYRVVSVLTVLHQDWLNGKEYKCKVSNKALPAPIEKTISKAKGQPREPQVYTLPPSRDELTKNQVSLVCLVKGFYPSDIAVEWESNGQPENNYKTTPPVLTSDGSFFLYSKLTVDKSRWQQGNVFSCSVMHEALHNHYTQKSLSLSPGK

SEQ ID NO: 21 - protein, 232 aa, Artificial
  Fc2 sequence
EPKSCDKTHTCPPCPAPELLGGPSVFLFPPKPKDTLMISRTPEVTCVVVDVSHEDPEVKFNWYVDGVEVHNAKTKPREEQYNSTYRVVSVLTVLHQDWLNGKEYKCKVSNKALPAPIEKTISKAKGQPREPQVYTKPPSRDELTKNQVSLTCLVKGFYPSDIAVEWESNGQPENNYKTTPPVLDSDGSFFLTSQLTVDKSRWQQGNVFSCSVMHEALHNHYTQKSLSLSPGK

SEQ ID NO: 22 - protein, 232 aa, Artificial
  Fc1 sequence
EPKSCDKTHTCPPCPAPELLGGPSVFLFPPKPKDTLMISRTPEVTCVVVDVSHEDPEVKFNWYVDGVEVHNAKTKPREEQYNSTYRVVSVLTVLHQDWLNGKEYKCKVSNKALPAPIEKTISKAKGQPREPQVYTLPPSRDELTKNQVSLLCLVKGFYPSDIAVEWESNGQPENNYKTTPPVLASDGSFFLYSKLTVDKSRWQQGNVFSCSVMHEALHNHYTQKSLSLSPGK

SEQ ID NO: 23 - protein, 232 aa, Artificial
  Fc2 sequence
EPKSCDKTHTCPPCPAPELLGGPSVFLFPPKPKDTLMISRTPEVTCVVVDVSHEDPEVKFNWYVDGVEVHNAKTKPREEQYNSTYRVVSVLTVLHQDWLNGKEYKCKVSNKALPAPIEKTISKAKGQPREPQVYTWPPSRDELTKNQVSLTCLVKGFYPSDIAVEWESNGQPENNYKTTPPVLDSDGSFFLHSRLTVDKSRWQQGNVFSCSVMHEALHNHYTQKSLSLSPGK

SEQ ID NO: 24 - protein, 232 aa, Artificial
  Fc1 sequence
EPKSCDKTHTCPPCPAPELLGGPSVFLFPPKPKDTLMISRTPEVTCVVVDVSHEDPEVKFNWYVDGVEVHNAKTKPREEQYNSTYRVVSVLTVLHQDWLNGKEYKCKVSNKALPAPIEKTISKAKGQPREPQVYTLPPSRDELTKNQVSLPCLVKGFYPSDIAVEWESNGQPENNYKTTPPVLNSDGSFFLYSKLTVDKSRWQQGNVFSCSVMHEALHNHYTQKSLSLSPGK

SEQ ID NO: 25 - protein, 232 aa, Artificial
  Fc2 sequence
EPKSCDKTHTCPPCPAPELLGGPSVFLFPPKPKDTLMISRTPEVTCVVVDVSHEDPEVKFNWYVDGVEVHNAKTKPREEQYNSTYRVVSVLTVLHQDWLNGKEYKCKVSNKALPAPIEKTISKAKGQPREPQVYTVPPSRDELTKNQVSLTCLVKGFYPSDIAVEWESNGQPENNYKTTPPVLDSDGSFFLPSSLTVDKSRWQQGNVFSCSVMHEALHNHYTQKSLSLSPGK

SEQ ID NO: 26 - protein, 232 aa, Artificial
  Fc1 sequence
EPKSCDKTHTCPPCPAPELLGGPSVFLFPPKPKDTLMISRTPEVTCVVVDVSHEDPEVKFNWYVDGVEVHNAKTKPREEQYNSTYRVVSVLTVLHQDWLNGKEYKCKVSNKALPAPIEKTISKAKGQPREPQVYTLPPSRDELTKNQVSLPCLVKGFYPSDIAVEWESNGQPENNYKTTPPVLISDGSFFLYSKLTVDKSRWQQGNVFSCSVMHEALHNHYTQKSLSLSPGK

SEQ ID NO: 27 - protein, 232 aa, Artificial
  Fc2 sequence
EPKSCDKTHTCPPCPAPELLGGPSVFLFPPKPKDTLMISRTPEVTCVVVDVSHEDPEVKFNWYVDGVEVHNAKTKPREEQYNSTYRVVSVLTVLHQDWLNGKEYKCKVSNKALPAPIEKTISKAKGQPREPQVYTPPPSRDELTKNQVSLTCLVKGFYPSDIAVEWESNGQPENNYKTTPPVLDSDGSFFLFSFLTVDKSRWQQGNVFSCSVMHEALHNHYTQKSLSLSPGK

SEQ ID NO: 28 - protein, 232 aa, Artificial
  Fc1 sequence
EPKSCDKTHTCPPCPAPELLGGPSVFLFPPKPKDTLMISRTPEVTCVVVDVSHEDPEVKFNWYVDGVEVHNAKTKPREEQYNSTYRVVSVLTVLHQDWLNGKEYKCKVSNKALPAPIEKTISKAKGQPREPQVYTLPPSRDELTKNQVSLWCLVKGFYPSDIAVEWESNGQPENNYKTTPPVLGSDGSFFLYSKLTVDKSRWQQGNVFSCSVMHEALHNHYTQKSLSLSPGK

SEQ ID NO: 29 - protein, 232 aa, Artificial
  Fc2 sequence
EPKSCDKTHTCPPCPAPELLGGPSVFLFPPKPKDTLMISRTPEVTCVVVDVSHEDPEVKFNWYVDGVEVHNAKTKPREEQYNSTYRVVSVLTVLHQDWLNGKEYKCKVSNKALPAPIEKTISKAKGQPREPQVYTDPPSRDELTKNQVSLTCLVKGFYPSDIAVEWESNGQPENNYKTTPPVLDSDGSFFLPSSLTVDKSRWQQGNVFSCSVMHEALHNHYTQKSLSLSPGK

SEQ ID NO: 30 - protein, 232 aa, Artificial
  Fc1 sequence
EPKSCDKTHTCPPCPAPELLGGPSVFLFPPKPKDTLMISRTPEVTCVVVDVSHEDPEVKFNWYVDGVEVHNAKTKPREEQYNSTYRVVSVLTVLHQDWLNGKEYKCKVSNKALPAPIEKTISKAKGQPREPQVYTLPPSRDELTKNQVSLLCLVKGFYPSDIAVEWESNGQPENNYKTTPPVLRSDGSFFLYSKLTVDKSRWQQGNVFSCSVMHEALHNHYTQKSLSLSPGK

SEQ ID NO: 31 - protein, 232 aa, Artificial
  Fc2 sequence
EPKSCDKTHTCPPCPAPELLGGPSVFLFPPKPKDTLMISRTPEVTCVVVDVSHEDPEVKFNWYVDGVEVHNAKTKPREEQYNSTYRVVSVLTVLHQDWLNGKEYKCKVSNKALPAPIEKTISKAKGQPREPQVYTEPPSRDELTKNQVSLTCLVKGFYPSDIAVEWESNGQPENNYKTTPPVLDSDGSFFLLSVLTVDKSRWQQGNVFSCSVMHEALHNHYTQKSLSLSPGK

SEQ ID NO: 32 - DNA, 312 bp, Artificial
  VL sequence
gacattcagatgactcagagcccttcttcactgtcagcttccgtgggcgacagagtcactatcacctgccgcgcaagtcaggatgtgaacaccgcagtcgcctggtaccagcagaagcctggcaaagctccaaagctgctgatctacagcgcatctttcctgtattctggagtgcccagtaggtttagtgggtcacggtccggtaccgacttcacactgactatctccagcctgcagcctgaggattttgccacatactattgccagcagcactataccacaccccctactttcggccagggaaccaaagtg

SEQ ID NO: 33 - protein, 104 aa, Artificial
  VL sequence
DIQMTQSPSSLSASVGDRVTITCRASQDVNTAVAWYQQKPGKAPKLLIYSASFLYSGVPSRFSGSRSGTDFTLTISSLQPEDFATYYCQQHYTTPPTFGQGTKV

SEQ ID NO: 34 - DNA, 330 bp, Artificial
  CL sequence
gagatcaagcgaactgtggccgctccaagcgtcttcatttttccaccctctgacgaacagctgaagtcagggacagcttccgtggtctgtctgctgaacaatttttaccccagggaggccaaagtgcagtggaaggtcgataacgctctgcagagcggaaattctcaggagagtgtgacagaacaggactcaaaagattccacttatagcctgtctagtaccctgacactgtccaaggcagactacgaaaagcataaagtgtatgcctgtgaggtcacacatcagggtctgtcaagccccgtcactaagtccttcaatcgtggcgaatgc

SEQ ID NO: 35 - protein, 110 aa, Artificial
  CL sequence
EIKRTVAAPSVFIFPPSDEQLKSGTASVVCLLNNFYPREAKVQWKVDNALQSGNSQESVTEQDSKDSTYSLSSTLTLSKADYEKHKVYACEVTHQGLSSPVTKSFNRGEC

SEQ ID NO: 36 - DNA, 360 bp, Artificial
  VH sequence
gaggtgcagctggtcgaaagtgggggtgggctggtgcagccaggcggatcactgaggctgtcctgcgccgctagcggcttcaacatcaaagacacctatattcactgggtccgacaggcaccagggaagggtctggaatgggtggctcgtatctaccctacaaatggttacactagatatgccgactccgtgaaaggccggtttactatttctgctgataccagtaagaacacagcatacctgcagatgaatagcctgagggctgaggataccgcagtgtactattgctctcggtgggggggtgacggcttctacgctatggattattggggccagggaactctggtcaccgtgtccagc

SEQ ID NO: 37 - protein, 120 aa, Artificial [sequence omitted]

SEQ ID NO: 38 - DNA, 990 bp, Artificial
  CH sequence
gcttcaacaaaaggaccttccgtgtttccactggcaccctctagtaagagtacttcaggaggaaccgcagcactgggatgtctggtgaaggactacttcccagagcccgtcaccgtgtcttggaacagtggagcactgacctccggggtccatacatttcctgccgtgctgcagtcatccggtctgtatagcctgagctctgtggtcacagtcccaagttcatccctgggcacccagacatacatctgcaacgtgaatcacaaaccttccaatactaaggtcgacaagaaagtggaaccaaaaagctgtgataagactcatacctgcccaccttgtcctgcaccagagctgctgggaggtccaagcgtgttcctgtttccacccaagcccaaagacacactgatgatttctcgcacacccgaagtcacttgtgtggtcgtggacgtgtcccacgaggatcctgaagtcaagttcaactggtacgtggatggcgtcgaggtgcataatgctaagaccaaacccagagaggaacagtacaacagcacctatcgcgtcgtgtctgtcctgacagtgctgcaccaggattggctgaacggaaaggagtacaagtgcaaagtgagcaacaaggccctgcccgctcctatcgagaagaccatttctaaggctaaaggccagcctagagaaccacaggtgtatacactgcctccaagtcgcgacgagctgacaaaaaaccaggtctccctgctgtgtctggtgaagggattctaccctagcgatatcgcagtggagtgggaatctaatgggcagccagaaaacaattataagaccacaccccctgtgctgtgctcagatggttccttctttctgtacagtaaactgaccgtggacaagtccaggtggcagcaggggaacgtcttttcctgcagcgtgatgcatgaggccctgcacaatcattacacacagaaatctctgagtctgtcaccaggaaag

SEQ ID NO: 39 - protein, 330 aa, Artificial
  CH sequence
ASTKGPSVFPLAPSSKSTSGGTAALGCLVKDYFPEPVTVSWNSGALTSGVHTFPAVLQSSGLYSLSSVVTVPSSSLGTQTYICNVNHKPSNTKVDKKVEPKSCDKTHTCPPCPAPELLGGPSVFLFPPKPKDTLMISRTPEVTCVVVDVSHEDPEVKFNWYVDGVEVHNAKTKPREEQYNSTYRVVSVLTVLHQDWLNGKEYKCKVSNKALPAPIEKTISKAKGQPREPQVYTLPPSRDELTKNQVSLLCLVKGFYPSDIAVEWESNGQPENNYKTTPPVLCSDGSFFLYSKLTVDKSRWQQGNVFSCSVMHEALHNHYTQKSLSLSPGK

SEQ ID NO: 40 - DNA, 990 bp, Artificial
  CH sequence
gcttcaacaaaaggaccttccgtgtttccactggcaccctctagtaagagtacttcaggaggaaccgcagcactgggatgtctggtgaaggactacttcccagagcccgtcaccgtgtcttggaacagtggagcactgacctccggggtccatacatttcctgccgtgctgcagtcatccggtctgtatagcctgagctctgtggtcacagtcccaagttcatccctgggcacccagacatacatctgcaacgtgaatcacaaaccttccaatactaaggtcgacaagaaagtggaaccaaaaagctgtgataagactcatacctgcccaccttgtcctgcaccagagctgctgggaggtccaagcgtgttcctgtttccacccaagcccaaagacacactgatgatttctcgcacacccgaagtcacttgtgtggtcgtggacgtgtcccacgaggatcctgaagtcaagttcaactggtacgtggatggcgtcgaggtgcataatgctaagaccaaacccagagaggaacagtacaacagcacctatcgcgtcgtgtctgtcctgacagtgctgcaccaggattggctgaacggaaaggagtacaagtgcaaagtgagcaacaaggccctgcccgctcctatcgagaagaccatttctaaggctaaaggccagcctagagaaccacaggtgtatacagagcctccaagtcgcgacgagctgacaaaaaaccaggtctccctgacttgtctggtgaagggattctaccctagcgatatcgcagtggagtgggaatctaatgggcagccagaaaacaattataagaccacaccccctgtgctggactcagatggttccttctttctgctgagtgtgctgaccgtggacaagtccaggtggcagcaggggaacgtcttttcctgcagcgtgatgcatgaggccctgcacaatcattacacacagaaatctctgagtctgtcaccaggaaag

SEQ ID NO: 41 - protein, 330 aa, Artificial
  CH sequence
ASTKGPSVFPLAPSSKSTSGGTAALGCLVKDYFPEPVTVSWNSGALTSGVHTFPAVLQSSGLYSLSSVVTVPSSSLGTQTYICNVNHKPSNTKVDKKVEPKSCDKTHTCPPCPAPELLGGPSVFLFPPKPKDTLMISRTPEVTCVVVDVSHEDPEVKFNWYVDGVEVHNAKTKPREEQYNSTYRVVSVLTVLHQDWLNGKEYKCKVSNKALPAPIEKTISKAKGQPREPQVYTEPPSRDELTKNQVSLTCLVKGFYPSDIAVEWESNGQPENNYKTTPPVLDSDGSFFLLSVLTVDKSRWQQGNVFSCSVMHEALHNHYTQKSLSLSPGK

SEQ ID NO: 42 - DNA, 309 bp, Artificial
  VL sequence
cagatcgtgctgagccagagccccgccatcctgagcgccagccccggcgagaaggtgaccatgacctgcagggccagcagcagcgtgagctacatccactggttccagcagaagcccggcagcagccccaagccctggatctacgccaccagcaacctggccagcggcgtgcccgtgaggttcagcggcagcggcagcggcaccagctacagcctgaccatcagcagggtggaggccgaggacgccgccacctactactgccagcagtggaccagcaacccccccaccttcggcggcggcaccaagctg

SEQ ID NO: 43 - protein, 103 aa, Artificial
  VL sequence
QIVLSQSPAILSASPGEKVTMTCRASSSVSYIHWFQQKPGSSPKPWIYATSNLASGVPVRFSGSGSGTSYSLTISRVEAEDAATYYCQQWTSNPPTFGGGTKL

SEQ ID NO: 44 - DNA, 363 bp, Artificial
  VH sequence
caggtgcagctgcagcagcccggcgccgagctggtgaagcccggcgccagcgtgaagatgagctgcaaggccagcggctacaccttcaccagctacaacatgcactgggtgaagcagacccccggcaggggcctggagtggatcggcgccatctaccccggcaacggcgacaccagctacaaccagaagttcaagggcaaggccaccctgaccgccgacaagagcagcagcaccgcctacatgcagctgagcagcctgaccagcgaggacagcgccgtgtactactgcgccaggagcacctactacggcggcgactggtacttcaacgtgtggggcgccggcaccaccgtgaccgtgagcgcc

SEQ ID NO: 45 - protein, 121 aa, Artificial [sequence omitted]

SEQ ID NO: 46 - DNA, 990 bp, Artificial; identical to SEQ ID NO: 38
  CH sequence

SEQ ID NO: 47 - DNA, 990 bp, Artificial
  CH sequence
gcttcaacaaaaggaccttccgtgtttccactggcaccctctagtaagagtacttcaggaggaaccgcagcactgggatgtctggtgaaggactacttcccagagcccgtcaccgtgtcttggaacagtggagcactgacctccggggtccatacatttcctgccgtgctgcagtcatccggtctgtatagcctgagctctgtggtcacagtcccaagttcatccctgggcacccagacatacatctgcaacgtgaatcacaaaccttccaatactaaggtcgacaagaaagtggaaccaaaaagctgtgataagactcatacctgcccaccttgtcctgcaccagagctgctgggaggtccaagcgtgttcctgtttccacccaagcccaaagacacactgatgatttctcgcacacccgaagtcacttgtgtggtcgtggacgtgtcccacgaggatcctgaagtcaagttcaactggtacgtggatggcgtcgaggtgcataatgctaagaccaaacccagagaggaacagtacaacagcacctatcgcgtcgtgtctgtcctgacagtgctgcaccaggattggctgaacggaaaggagtacaagtgcaaagtgagcaacaaggccctgcccgctcctatcgagaagaccatttctaaggctaaaggccagcctagagaaccacaggtgtatacactgcctccaagtcgcgacgagctgacaaaaaaccaggtctccctgctgtgtctggtgaagggattctaccctagcgatatcgcagtggagtgggaatctaatgggcagccagaaaacaattataagaccacaccccctgtgctgcggtcagatggttccttctttctgtacagtaaactgaccgtggacaagtccaggtggcagcaggggaacgtcttttcctgcagcgtgatgcatgaggccctgcacaatcattacacacagaaatctctgagtctgtcaccaggaaag

SEQ ID NO: 48 - protein, 330 aa, Artificial; identical to SEQ ID NO: 39
  CH sequence

SEQ ID NO: 49 - protein, 330 aa, Artificial
  CH sequence
ASTKGPSVFPLAPSSKSTSGGTAALGCLVKDYFPEPVTVSWNSGALTSGVHTFPAVLQSSGLYSLSSVVTVPSSSLGTQTYICNVNHKPSNTKVDKKVEPKSCDKTHTCPPCPAPELLGGPSVFLFPPKPKDTLMISRTPEVTCVVVDVSHEDPEVKFNWYVDGVEVHNAKTKPREEQYNSTYRVVSVLTVLHQDWLNGKEYKCKVSNKALPAPIEKTISKAKGQPREPQVYTLPPSRDELTKNQVSLLCLVKGFYPSDIAVEWESNGQPENNYKTTPPVLRSDGSFFLYSKLTVDKSRWQQGNVFSCSVMHEALHNHYTQKSLSLSPGK

SEQ ID NO: 50 - DNA, 312 bp, Artificial
  VL sequence
gatatccagctgacccagagccctagcagcctgagcgctagcgtgggcgacagggtgagcatcacctgcaaggccagccaggacgtgtccatcgccgtggcctggtatcaacagaagcccggcaaggcccccaagctgctgatctacagcgccagctacaggtacaccggcgtgcccgacagatttagcggcagcggctccggcacagacttcaccctgaccatcagcagcctgcagcccgaggacttcgccgtgtactactgccagcagcactacatcacccccctgacctttggcgccggcaccaaagtg

SEQ ID NO: 51 - protein, 104 aa, Artificial
  VL sequence
DIQLTQSPSSLSASVGDRVSITCKASQDVSIAVAWYQQKPGKAPKLLIYSASYRYTGVPDRFSGSGSGTDFTLTISSLQPEDFAVYYCQQHYITPLTFGAGTKV

SEQ ID NO: 52 - DNA, 360 bp, Artificial
  VH sequence
gtgcagctgcagcagtccggcagcgagctgaagaagcctggcgccagcgtgaaggtgagctgcaaggccagcggctacaccttcaccaactacggcatgaactgggtgaagcaggcccctggccagggactgaagtggatgggctggatcaacacctacaccggcgagcccacctacaccgacgacttcaagggcaggttcgccttcagcctggacaccagcgtgtccaccgcctacctgcagatctccagcctgaaggccgacgacaccgccgtgtacttctgcgccagaggcggcttcggcagcagctactggtacttcgacgtgtggggccagggaagcctggtgaccgtgagcagc

SEQ ID NO: 53 - protein, 120 aa, Artificial
  VH sequence
VQLQQSGSELKKPGASVKVSCKASGYTFTNYGMNWVKQAPGQGLKWMGWINTYTGEPTYTDDFKGRFAFSLDTSVSTAYLQISSLKADDTAVYFCARGGFGSSYWYFDVWGQGSLVTVSS

SEQ ID NO: 54 - DNA, 990 bp, Artificial
  CH sequence
gcttcaacaaaaggaccttccgtgtttccactggcaccctctagtaagagtacttcaggaggaaccgcagcactgggatgtctggtgaaggactacttcccagagcccgtcaccgtgtcttggaacagtggagcactgacctccggggtccatacatttcctgccgtgctgcagtcatccggtctgtatagcctgagctctgtggtcacagtcccaagttcatccctgggcacccagacatacatctgcaacgtgaatcacaaaccttccaatactaaggtcgacaagaaagtggaaccaaaaagctgtgataagactcatacctgcccaccttgtcctgcaccagagctgctgggaggtccaagcgtgttcctgtttccacccaagcccaaagacacactgatgatttctcgcacacccgaagtcacttgtgtggtcgtggacgtgtcccacgaggatcctgaagtcaagttcaactggtacgtggatggcgtcgaggtgcataatgctaagaccaaacccagagaggaacagtacaacagcacctatcgcgtcgtgtctgtcctgacagtgctgcaccaggattggctgaacggaaaggagtacaagtgcaaagtgagcaacaaggccctgcccgctcctatcgagaagaccatttctaaggctaaaggccagcctagagaaccacaggtgtatacactgcctccaagtcgcgacgagctgacaaaaaaccaggtctccctgccctgtctggtgaagggattctaccctagcgatatcgcagtggagtgggaatctaatgggcagccagaaaacaattataagaccacaccccctgtgctgaactcagatggttccttctttctgtacagtaaactgaccgtggacaagtccaggtggcagcaggggaacgtcttttcctgcagcgtgatgcatgaggccctgcacaatcattacacacagaaatctctgagtctgtcaccaggaaag

SEQ ID NO: 55 - protein, 330 aa, Artificial
  CH sequence
ASTKGPSVFPLAPSSKSTSGGTAALGCLVKDYFPEPVTVSWNSGALTSGVHTFPAVLQSSGLYSLSSVVTVPSSSLGTQTYICNVNHKPSNTKVDKKVEPKSCDKTHTCPPCPAPELLGGPSVFLFPPKPKDTLMISRTPEVTCVVVDVSHEDPEVKFNWYVDGVEVHNAKTKPREEQYNSTYRVVSVLTVLHQDWLNGKEYKCKVSNKALPAPIEKTISKAKGQPREPQVYTLPPSRDELTKNQVSLPCLVKGFYPSDIAVEWESNGQPENNYKTTPPVLNSDGSFFLYSKLTVDKSRWQQGNVFSCSVMHEALHNHYTQKSLSLSPGK

SEQ ID NO: 56 - DNA, 312 bp, Artificial
  VL sequence
gacatccagatgacccagagccctagcagcctgagcgctagcgtgggcgacagggtgaccatcacctgcagggccagccaggatgtgagcaccgctgtggcctggtatcaacagaagcccggcaaggcccccaagctgctgatctacagcgccagcttcctgtacagcggcgtgcccagcagatttagcggcagcggcagcggcaccgatttcaccctgaccatcagcagcctgcagcccgaggacttcgccacctactactgccagcagtacctgtaccatcccgccaccttcggccagggcaccaaggtg

SEQ ID NO: 57 - protein, 104 aa, Artificial
  VL sequence
DIQMTQSPSSLSASVGDRVTITCRASQDVSTAVAWYQQKPGKAPKLLIYSASFLYSGVPSRFSGSGSGTDFTLTISSLQPEDFATYYCQQYLYHPATFGQGTKV

SEQ ID NO: 58 - DNA, 354 bp, Artificial
  VH sequence
gaggtgcagctggtggagagcggaggaggactggtgcagcctggaggatccctgagactgagctgcgccgccagcggcttcaccttcagcgacagctggatccactgggtgagacaggcccctggcaagggcctggaatgggtggcctggatctccccttacggcggcagcacctactacgccgacagcgtgaagggcaggttcaccatcagcgccgacaccagcaagaacaccgcctacctgcagatgaacagcctgagggccgaggacaccgccgtgtactactgcgccagaagacactggcccggcggattcgactactggggacagggcaccctggtgaccgtgagcgcc

SEQ ID NO: 59 - protein, 118 aa, Artificial
  VH sequence
EVQLVESGGGLVQPGGSLRLSCAASGFTFSDSWIHWVRQAPGKGLEWVAWISPYGGSTYYADSVKGRFTISADTSKNTAYLQMNSLRAEDTAVYYCARRHWPGGFDYWGQGTLVTVSA

SEQ ID NO: 60 - DNA, 990 bp, Artificial
  CH sequence
gcttcaacaaaaggaccttccgtgtttccactggcaccctctagtaagagtacttcaggaggaaccgcagcactgggatgtctggtgaaggactacttcccagagcccgtcaccgtgtcttggaacagtggagcactgacctccggggtccatacatttcctgccgtgctgcagtcatccggtctgtatagcctgagctctgtggtcacagtcccaagttcatccctgggcacccagacatacatctgcaacgtgaatcacaaaccttccaatactaaggtcgacaagaaagtggaaccaaaaagctgtgataagactcatacctgcccaccttgtcctgcaccagagctgctgggaggtccaagcgtgttcctgtttccacccaagcccaaagacacactgatgatttctcgcacacccgaagtcacttgtgtggtcgtggacgtgtcccacgaggatcctgaagtcaagttcaactggtacgtggatggcgtcgaggtgcataatgctaagaccaaacccagagaggaacagtacaacagcacctatcgcgtcgtgtctgtcctgacagtgctgcaccaggattggctgaacggaaaggagtacaagtgcaaagtgagcaacaaggccctgcccgctcctatcgagaagaccatttctaaggctaaaggccagcctagagaaccacaggtgtatacactgcctccaagtcgcgacgagctgacaaaaaaccaggtctccctgtggtgtctggtgaagggattctaccctagcgatatcgcagtggagtgggaatctaatgggcagccagaaaacaattataagaccacaccccctgtgctgggatcagatggttccttctttctgtacagtaaactgaccgtggacaagtccaggtggcagcaggggaacgtcttttcctgcagcgtgatgcatgaggccctgcacaatcattacacacagaaatctctgagtctgtcaccaggaaag

SEQ ID NO: 61 - protein, 330 aa, Artificial
  CH sequence
ASTKGPSVFPLAPSSKSTSGGTAALGCLVKDYFPEPVTVSWNSGALTSGVHTFPAVLQSSGLYSLSSVVTVPSSSLGTQTYICNVNHKPSNTKVDKKVEPKSCDKTHTCPPCPAPELLGGPSVFLFPPKPKDTLMISRTPEVTCVVVDVSHEDPEVKFNWYVDGVEVHNAKTKPREEQYNSTYRVVSVLTVLHQDWLNGKEYKCKVSNKALPAPIEKTISKAKGQPREPQVYTLPPSRDELTKNQVSLWCLVKGFYPSDIAVEWESNGQPENNYKTTPPVLGSDGSFFLYSKLTVDKSRWQQGNVFSCSVMHEALHNHYTQKSLSLSPGK

SEQ ID NO: 62 - DNA, 729 bp, Artificial
  variable region sequence
gatatcaagctgcagcagagcggtgcagaactggccagacctggcgcttcagtgaaaatgtcctgtaagactagcggctacacattcactcgatataccatgcactgggtgaagcagcgtccagggcagggtctggagtggatcggatatattaacccctctcgcgggtacaccaactataatcagaagtttaaagacaaggccacactgactaccgataagagctctagtactgcttacatgcagctgtcatccctgaccagcgaagactctgcagtgtactattgcgcccgatactatgacgatcattactgtctggactactggggccagggaacaactctgactgtcagctctgtggagggaggaagtggaggttcaggaggatccggaggtagcggaggagtggacgatatccagctgacccagtctcccgccattatgtccgctagccctggcgagaaagtcaccatgacatgcagagccagttcatccgtgtcctacatgaattggtatcagcagaaatctggaacaagtccaaagaggtggatctacgacacttctaaggtcgcaagtggggtgccctatcggttttctgggagtggttcaggcacttcctacagcctgaccattagctctatggaggccgaagatgctgcaacctactattgccagcagtggagtagcaatcctctgacatttggagcagggactaaactggaactgaag

SEQ ID NO: 63 - protein, 243 aa, Artificial
  variable region sequence
DIKLQQSGAELARPGASVKMSCKTSGYTFTRYTMHWVKQRPGQGLEWIGYINPSRGYTNYNQKFKDKATLTTDKSSSTAYMQLSSLTSEDSAVYYCARYYDDHYCLDYWGQGTTLTVSSVEGGSGGSGGSGGSGGVDDIQLTQSPAIMSASPGEKVTMTCRASSSVSYMNWYQQKSGTSPKRWIYDTSKVASGVPYRFSGSGSGTSYSLTISSMEAEDAATYYCQQWSSNPLTFGAGTKLELK

SEQ ID NO: 64 - DNA, 990 bp, Artificial
  constant region sequence
gcttcaacaaaaggaccttccgtgtttccactggcaccctctagtaagagtacttcaggaggaaccgcagcactgggatgtctggtgaaggactacttcccagagcccgtcaccgtgtcttggaacagtggagcactgacctccggggtccatacatttcctgccgtgctgcagtcatccggtctgtatagcctgagctctgtggtcacagtcccaagttcatccctgggcacccagacatacatctgcaacgtgaatcacaaaccttccaatactaaggtcgacaagaaagtggaaccaaaaagctgtgataagactcatacctgcccaccttgtcctgcaccagagctgctgggaggtccaagcgtgttcctgtttccacccaagcccaaagacacactgatgatttctcgcacacccgaagtcacttgtgtggtcgtggacgtgtcccacgaggatcctgaagtcaagttcaactggtacgtggatggcgtcgaggtgcataatgctaagaccaaacccagagaggaacagtacaacagcacctatcgcgtcgtgtctgtcctgacagtgctgcaccaggattggctgaacggaaaggagtacaagtgcaaagtgagcaacaaggccctgcccgctcctatcgagaagaccatttctaaggctaaaggccagcctagagaaccacaggtgtatacaggacctccaagtcgcgacgagctgacaaaaaaccaggtctccctgacttgtctggtgaagggattctaccctagcgatatcgcagtggagtgggaatctaatgggcagccagaaaacaattataagaccacaccccctgtgctggactcagatggttccttctttctgctcagttgtctgaccgtggacaagtccaggtggcagcaggggaacgtcttttcctgcagcgtgatgcatgaggccctgcacaatcattacacacagaaatctctgagtctgtcaccaggaaag

SEQ ID NO: 65 - DNA, 990 bp, Artificial
  constant region sequence
gcttcaacaaaaggaccttccgtgtttccactggcaccctctagtaagagtacttcaggaggaaccgcagcactgggatgtctggtgaaggactacttcccagagcccgtcaccgtgtcttggaacagtggagcactgacctccggggtccatacatttcctgccgtgctgcagtcatccggtctgtatagcctgagctctgtggtcacagtcccaagttcatccctgggcacccagacatacatctgcaacgtgaatcacaaaccttccaatactaaggtcgacaagaaagtggaaccaaaaagctgtgataagactcatacctgcccaccttgtcctgcaccagagctgctgggaggtccaagcgtgttcctgtttccacccaagcccaaagacacactgatgatttctcgcacacccgaagtcacttgtgtggtcgtggacgtgtcccacgaggatcctgaagtcaagttcaactggtacgtggatggcgtcgaggtgcataatgctaagaccaaacccagagaggaacagtacaacagcacctatcgcgtcgtgtctgtcctgacagtgctgcaccaggattggctgaacggaaaggagtacaagtgcaaagtgagcaacaaggccctgcccgctcctatcgagaagaccatttctaaggctaaaggccagcctagagaaccacaggtgtatacatatcctccaagtcgcgacgagctgacaaaaaaccaggtctccctgacttgtctggtgaagggattctaccctagcgatatcgcagtggagtgggaatctaatgggcagccagaaaacaattataagaccacaccccctgtgctggactcagatggttccttctttctggcaagtcctctgaccgtggacaagtccaggtggcagcaggggaacgtcttttcctgcagcgtgatgcatgaggccctgcacaatcattacacacagaaatctctgagtctgtcaccaggaaag

SEQ ID NO: 66 - DNA, 990 bp, Artificial
  constant region sequence
gcttcaacaaaaggaccttccgtgtttccactggcaccctctagtaagagtacttcaggaggaaccgcagcactgggatgtctggtgaaggactacttcccagagcccgtcaccgtgtcttggaacagtggagcactgacctccggggtccatacatttcctgccgtgctgcagtcatccggtctgtatagcctgagctctgtggtcacagtcccaagttcatccctgggcacccagacatacatctgcaacgtgaatcacaaaccttccaatactaaggtcgacaagaaagtggaaccaaaaagctgtgataagactcatacctgcccaccttgtcctgcaccagagctgctgggaggtccaagcgtgttcctgtttccacccaagcccaaagacacactgatgatttctcgcacacccgaagtcacttgtgtggtcgtggacgtgtcccacgaggatcctgaagtcaagttcaactggtacgtggatggcgtcgaggtgcataatgctaagaccaaacccagagaggaacagtacaacagcacctatcgcgtcgtgtctgtcctgacagtgctgcaccaggattggctgaacggaaaggagtacaagtgcaaagtgagcaacaaggccctgcccgctcctatcgagaagaccatttctaaggctaaaggccagcctagagaaccacaggtgtatacagttcctccaagtcgcgacgagctgacaaaaaaccaggtctccctgacttgtctggtgaagggattctaccctagcgatatcgcagtggagtgggaatctaatgggcagccagaaaacaattataagaccacaccccctgtgctggactcagatggttccttctttctgccaagttcactgaccgtggacaagtccaggtggcagcaggggaacgtcttttcctgcagcgtgatgcatgaggccctgcacaatcattacacacagaaatctctgagtctgtcaccaggaaag

SEQ ID NO: 67 - DNA, 990 bp, Artificial
  constant region sequence
gcttcaacaaaaggaccttccgtgtttccactggcaccctctagtaagagtacttcaggaggaaccgcagcactgggatgtctggtgaaggactacttcccagagcccgtcaccgtgtcttggaacagtggagcactgacctccggggtccatacatttcctgccgtgctgcagtcatccggtctgtatagcctgagctctgtggtcacagtcccaagttcatccctgggcacccagacatacatctgcaacgtgaatcacaaaccttccaatactaaggtcgacaagaaagtggaaccaaaaagctgtgataagactcatacctgcccaccttgtcctgcaccagagctgctgggaggtccaagcgtgttcctgtttccacccaagcccaaagacacactgatgatttctcgcacacccgaagtcacttgtgtggtcgtggacgtgtcccacgaggatcctgaagtcaagttcaactggtacgtggatggcgtcgaggtgcataatgctaagaccaaacccagagaggaacagtacaacagcacctatcgcgtcgtgtctgtcctgacagtgctgcaccaggattggctgaacggaaaggagtacaagtgcaaagtgagcaacaaggccctgcccgctcctatcgagaagaccatttctaaggctaaaggccagcctagagaaccacaggtgtatacagatcctccaagtcgcgacgagctgacaaaaaaccaggtctccctgacttgtctggtgaagggattctaccctagcgatatcgcagtggagtgggaatctaatgggcagccagaaaacaattataagaccacaccccctgtgctggactcagatggttccttctttctgccaagtagtctgaccgtggacaagtccaggtggcagcaggggaacgtcttttcctgcagcgtgatgcatgaggccctgcacaatcattacacacagaaatctctgagtctgtcaccaggaaag

SEQ ID NO: 68 - protein, 330 aa, Artificial
  constant region sequence
ASTKGPSVFPLAPSSKSTSGGTAALGCLVKDYFPEPVTVSWNSGALTSGVHTFPAVLQSSGLYSLSSVVTVPSSSLGTQTYICNVNHKPSNTKVDKKVEPKSCDKTHTCPPCPAPELLGGPSVFLFPPKPKDTLMISRTPEVTCVVVDVSHEDPEVKFNWYVDGVEVHNAKTKPREEQYNSTYRVVSVLTVLHQDWLNGKEYKCKVSNKALPAPIEKTISKAKGQPREPQVYTGPPSRDELTKNQVSLTCLVKGFYPSDIAVEWESNGQPENNYKTTPPVLDSDGSFFLLSCLTVDKSRWQQGNVFSCSVMHEALHNHYTQKSLSLSPGK

SEQ ID NO: 69 - protein, 330 aa, Artificial
  constant region sequence
ASTKGPSVFPLAPSSKSTSGGTAALGCLVKDYFPEPVTVSWNSGALTSGVHTFPAVLQSSGLYSLSSVVTVPSSSLGTQTYICNVNHKPSNTKVDKKVEPKSCDKTHTCPPCPAPELLGGPSVFLFPPKPKDTLMISRTPEVTCVVVDVSHEDPEVKFNWYVDGVEVHNAKTKPREEQYNSTYRVVSVLTVLHQDWLNGKEYKCKVSNKALPAPIEKTISKAKGQPREPQVYTYPPSRDELTKNQVSLTCLVKGFYPSDIAVEWESNGQPENNYKTTPPVLDSDGSFFLASPLTVDKSRWQQGNVFSCSVMHEALHNHYTQKSLSLSPGK

SEQ ID NO: 70 - protein, 330 aa, Artificial
  constant region sequence
ASTKGPSVFPLAPSSKSTSGGTAALGCLVKDYFPEPVTVSWNSGALTSGVHTFPAVLQSSGLYSLSSVVTVPSSSLGTQTYICNVNHKPSNTKVDKKVEPKSCDKTHTCPPCPAPELLGGPSVFLFPPKPKDTLMISRTPEVTCVVVDVSHEDPEVKFNWYVDGVEVHNAKTKPREEQYNSTYRVVSVLTVLHQDWLNGKEYKCKVSNKALPAPIEKTISKAKGQPREPQVYTVPPSRDELTKNQVSLTCLVKGFYPSDIAVEWESNGQPENNYKTTPPVLDSDGSFFLPSSLTVDKSRWQQGNVFSCSVMHEALHNHYTQKSLSLSPGK

SEQ ID NO: 71 - protein, 330 aa, Artificial
  constant region sequence
ASTKGPSVFPLAPSSKSTSGGTAALGCLVKDYFPEPVTVSWNSGALTSGVHTFPAVLQSSGLYSLSSVVTVPSSSLGTQTYICNVNHKPSNTKVDKKVEPKSCDKTHTCPPCPAPELLGGPSVFLFPPKPKDTLMISRTPEVTCVVVDVSHEDPEVKFNWYVDGVEVHNAKTKPREEQYNSTYRVVSVLTVLHQDWLNGKEYKCKVSNKALPAPIEKTISKAKGQPREPQVYTDPPSRDELTKNQVSLTCLVKGFYPSDIAVEWESNGQPENNYKTTPPVLDSDGSFFLPSSLTVDKSRWQQGNVFSCSVMHEALHNHYTQKSLSLSPGK

SEQ ID NO: 72 - protein, 15 aa, Artificial
  Synthetic
GGGGSGGGGSGGGGS

SEQ ID NO: 73 - protein, 213 aa, Artificial
  Anti-CD20 light chain in anti-CD20 homodimer
QIVLSQSPAILSASPGEKVTMTCRASSSVSYIHWFQQKPGSSPKPWIYATSNLASGVPVRFSGSGSGTSYSLTISRVEAEDAATYYCQQWTSNPPTFGGGTKLEIKRTVAAPSVFIFPPSDEQLKSGTASVVCLLNNFYPREAKVQWKVDNALQSGNSQESVTEQDSKDSTYSLSSTLTLSKADYEKHKVYACEVTHQGLSSPVTKSFNRGEC

SEQ ID NO: 74 - protein, 451 aa, Artificial
  Anti-CD20 heavy chain in anti-CD20 homodimer
QVQLQQPGAELVKPGASVKMSCKASGYTFTSYNMHWVKQTPGRGLEWIGAIYPGNGDTSYNQKFKGKATLTADKSSSTAYMQLSSLTSEDSAVYYCARSTYYGGDWYFNVWGAGTTVTVSAASTKGPSVFPLAPSSKSTSGGTAALGCLVKDYFPEPVTVSWNSGALTSGVHTFPAVLQSSGLYSLSSVVTVPSSSLGTQTYICNVNHKPSNTKVDKKVEPKSCDKTHTCPPCPAPELLGGPSVFLFPPKPKDTLMISRTPEVTCVVVDVSHEDPEVKFNWYVDGVEVHNAKTKPREEQYNSTYRVVSVLTVLHQDWLNGKEYKCKVSNKALPAPIEKTISKAKGQPREPQVYTLPPSRDELTKNQVSLLCLVKGFYPSDIAVEWESNGQPENNYKTTPPVLRSDGSFFLYSKLTVDKSRWQQGNVFSCSVMHEALHNHYTQKSLSLSPGK

SEQ ID NO: 75 - protein, 214 aa, Artificial
  Anti-HER2 light chain in anti-HER2 homodimer
DIQMTQSPSSLSASVGDRVTITCRASQDVNTAVAWYQQKPGKAPKLLIYSASFLYSGVPSRFSGSRSGTDFTLTISSLQPEDFATYYCQQHYTTPPTFGQGTKVEIKRTVAAPSVFIFPPSDEQLKSGTASVVCLLNNFYPREAKVQWKVDNALQSGNSQESVTEQDSKDSTYSLSSTLTLSKADYEKHKVYACEVTHQGLSSPVTKSFNRGEC

SEQ ID NO: 76 - protein, 450 aa, Artificial
  Anti-HER2 heavy chain in anti-HER2 homodimer
EVQLVESGGGLVQPGGSLRLSCAASGFNIKDTYIHWVRQAPGKGLEWVARIYPTNGYTRYADSVKGRFTISADTSKNTAYLQMNSLRAEDTAVYYCSRWGGDGFYAMDYWGQGTLVTVSSASTKGPSVFPLAPSSKSTSGGTAALGCLVKDYFPEPVTVSWNSGALTSGVHTFPAVLQSSGLYSLSSVVTVPSSSLGTQTYICNVNHKPSNTKVDKKVEPKSCDKTHTCPPCPAPELLGGPSVFLFPPKPKDTLMISRTPEVTCVVVDVSHEDPEVKFNWYVDGVEVHNAKTKPREEQYNSTYRVVSVLTVLHQDWLNGKEYKCKVSNKALPAPIEKTISKAKGQPREPQVYTEPPSRDELTKNQVSLTCLVKGFYPSDIAVEWESNGQPENNYKTTPPVLDSDGSFFLLSVLTVDKSRWQQGNVFSCSVMHEALHNHYTQKSLSLSPGK

SEQ ID NO: 77 - protein, 213 aa, Artificial; identical to SEQ ID NO: 73
  Anti-CD20 light chain in anti-CD20/HER2 heterodimer

SEQ ID NO: 78 - protein, 451 aa, Artificial; identical to SEQ ID NO: 74
  Anti-CD20 heavy chain in anti-CD20/HER2 heterodimer

SEQ ID NO: 79 - protein, 214 aa, Artificial; identical to SEQ ID NO: 75
  Anti-HER2 light chain in anti-CD20/HER2 heterodimer

SEQ ID NO: 80 - protein, 450 aa, Artificial; identical to SEQ ID NO: 76
  Anti-HER2 heavy chain in anti-CD20/HER2 heterodimer